European Patent Specification EP 4 037 469 B1, published April 15, 2026. Title: Bacterial preparations for ice nucleation. Applicant: Logon Patentverwertungs-Verwaltungs GmbH. The sequence listing filed with the application follows.

SEQUENCE LISTING (15 sequences)

SEQ ID NO: 1 - DNA, 3603 bp, Pseudomonas syringae
atgaatctcgacaaggcgttggtgctgcgtacctgtgcaaataacatggccgatcactgcggccttatatggcccgcgtccggcacggtggaatccagatactggcagtcaaccaggcggcatgagaatggtctggtcggtttactgtggggcgctggaaccagcgcttttctaagcgtgcatgccgatgctcgatggattgtctgtgaagttgccgttgcagacatcatcagtctggaagagccgggaatggtcaagtttccgcgggccgaggtggttcatgtcggcgacaggatcagcgcgtcacacttcatttcggcacgtcaggccgaccctgcgtcaacatcaacatcaacgttaacgccaatgcccactgccatacccacgcccatgcctgccgtagcaagtgtcacgttaccggtggccgaacaggcccgtcatgaagtgttcgatgtcgcgtcggtcagcgcggctgccgccccagtaaacaccctgccggtgacgacgccgcagaatgtgcagaccgccacttacggcagcacgttgagtggcgacaatcacagtcgtctgattgccggttatggcagtaacgagaccgctggcaaccacagtgatctaattgccggttatggaagtacaggcaccgccggctccgacagctggctggtcgctggctatggaagcacccagaccgccggtggggacagcgcgctgacagcgggttacggcagcacccagaccgcccgcgaaggcagcaacctgacggcagggtacggcagcaccggcacggcaggctcggacagttcgctgatcgccggttacggcagtactcagacttcgggcggggacagctcactcacagcgggttacggcagcacgcaaacggctcaggaaggcagcaatctcaccgctgggtatggcagcaccggcacggcaggctcggacagctcgttgatcgccggttatggcagtacacaaacctcgggaggcgacagttcgctgaccgcgggctacggcagtacgcagacggcccaggagggcagcaatctgacggcggggtacggcagcacgggtacagcaggtgtcgacagctctctgatcgcgggatacggcagcacgcagacctcgggaagtgacagcgccctgaccgcaggctatggcagcacgcaaacggcccaggaaggcagcaatctcactgctgggtatggcagcaccggcacggcaggttccgacagctcgctgatcgccggttacggcagcacgcaaacctcgggcagtgacagctcgctcacggcggggtacggcagtacgcagacggctcaggaaggcagcaatctgacggcggggtacggcagcacgggtacagcaggtgtcgacagttcgttgatcgccggatatggcagcacgcagacctcgggaagtgacagtgcgctgacagcgggttacggcagcacgcaaacggcccaggaaggcagcaacctgacggcgggctacggcagcactggcacggcaggtgccgacagttcgttgatcgccggatatggcagcacgcagacgtcaggcagcgaaagttcgcttaccgcaggctatggcagtacccagactgcccgtgagggcagcaccctgacggccggatatggcagtaccggaacagctggcgctgacagctcgctgatcgccggttacggcagcacgcaaacctcgggcagtgaaagctcgctcacggcaggttatggcagtacccagaccgcacagcagggcagcgtactcacatcaggctatggcagtacgcaaacggccggggctgccagtaacctcaccaccggttacggaagtacaggtaccgcaggtcacgagagtttcatcattgcgggttatggaagtacacagacagcgggccacaaaagtatcctgaccgctggttatggcagtactcagacggccagggacggtagcgacctgattgcgggctatggcagtacgggaaccgcaggctcgggcagttcgctgatcgcaggttatggcagcacccagaccgcgagttacagaagcatgctgaccgccggttatggcagtacccagaccgccagagaacacagcgaccttgtcacaggctatggcagcacttcaacggcagggtcaaacagttcgctgatcgccggctatggaagcactcagacggcgggcttcaaaagcatactgaccgccggttacggcagtacccagacggcacaggagcgcagcgacctggtcgcaggctacggaagcacgtcgactgcgggctattccagttccttgatcgccggctatggcagcacgcagacggcaggctacgaaagcacgttgaccgccggttacggcagtacgcaaaccgctcaggaaaacagctcgctcaccacaggttacggaagtacttctactgcgggctattccagctcgctcatcgcgggttacggcagtacgcaaacggcaggctacgagagcacgttgaccgccggttacggtagtacgcaaaccgcgaaggagcgcagtgatctggtgacaggttatggaagtacctccaccgccggctatgcgagctcgctgattgcgggttatggcagcacgcagactgcgggttatgagagcacgttgaccgccggttacggcagcacgcaaaccgcacaggaaaacagctcgctcaccaccgggtacggaagtacctccacagccggctttgccagctcgctgatcgccggttatggcagtacgcagacagccggctataaaagtaccctcacggccggttacggcagtactcagaccgcagagtatggaagctcactcactgcgggctacggcagcactgcaacggccgggcaggacagttcattgatagccggctatggcagctccctgaccagcggaatcagaagttttctgacggcaggctatggcagtacgctgatcgccggacttcgcagcgttttgatcgccggttatggcagtagtcttacatcgggcgttcgcagcacgttgactgcgggttatggcagtaaccagattgcaagttacggcagctcgttgattgcaggccatgaaagcattcaggtcgccggaaataaaagcatgctgatcgccggcaagggcagctcgcagacagcaggttttcgcagcacgctgattgccggtgcgggcagtgtacaactggcgggtgatcgcagccggttgattgccggtgcagacagtaatcagaccgcgggtgaccgcagcaaactgctggccggtaataacagttatctgactgccggcgatagaagcaaactgaccggcgggcatgactgcaccctgatggcgggagaccaaagcagattgaccgctggtaagaacagtgtcttgacggcaggcgctcgtagcaaactgattggcagtgaaggctcgacgctctcggctggagaagactccatacttattttcaggctctgggacgggaagaggtacaggcaactggtcgccagaacgggtgagaacggtgttgaggccgacataccgtattacgtgaacgaagatgacgatattgtcgataaacccgacgaggacgatgactggatagaggtaaagtag

SEQ ID NO: 2 - DNA, 3121 bp, Pseudomonas syringae
agtaaacaccctgccggtgacgacgccgcagaatgtgcagaccgccacttacggcagcacgttgagtggcgacaatcacagtcgtctgattgccggttatggcagtaacgagaccgctggcaaccacagtgatctaattgccggttatggaagtacaggcaccgccggctccgacagctggctggtcgctggctatggaagcacccagaccgccggtggggacagcgcgctgacagcgggttacggcagcacccagaccgcccgcgaaggcagcaacctgacggcagggtacggcagcaccggcacggcaggctcggacagttcgctgatcgccggttacggcagtactcagacttcgggcggggacagctcactcacagcgggttacggcagcacgcaaacggctcaggaaggcagcaatctcaccgctgggtatggcagcaccggcacggcaggctcggacagctcgttgatcgccggttatggcagtacacaaacctcgggaggcgacagttcgctgaccgcgggctacggcagtacgcagacggcccaggagggcagcaatctgacggcggggtacggcagcacgggtacagcaggtgtcgacagctctctgatcgcgggatacggcagcacgcagacctcgggaagtgacagcgccctgaccgcaggctatggcagcacgcaaacggcccaggaaggcagcaatctcactgctgggtatggcagcaccggcacggcaggttccgacagctcgctgatcgccggttacggcagcacgcaaacctcgggcagtgacagctcgctcacggcggggtacggcagtacgcagacggctcaggaaggcagcaatctgacggcggggtacggcagcacgggtacagcaggtgtcgacagttcgttgatcgccggatatggcagcacgcagacctcgggaagtgacagtgcgctgacagcgggttacggcagcacgcaaacggcccaggaaggcagcaacctgacggcgggctacggcagcactggcacggcaggtgccgacagttcgttgatcgccggatatggcagcacgcagacgtcaggcagcgaaagttcgcttaccgcaggctatggcagtacccagactgcccgtgagggcagcaccctgacggccggatatggcagtaccggaacagctggcgctgacagctcgctgatcgccggttacggcagcacgcaaacctcgggcagtgaaagctcgctcacggcaggttatggcagtacccagaccgcacagcagggcagcgtactcacatcaggctatggcagtacgcaaacggccggggctgccagtaacctcaccaccggttacggaagtacaggtaccgcaggtcacgagagtttcatcattgcgggttatggaagtacacagacagcgggccacaaaagtatcctgaccgctggttatggcagtactcagacggccagggacggtagcgacctgattgcgggctatggcagtacgggaaccgcaggctcgggcagttcgctgatcgcaggttatggcagcacccagaccgcgagttacagaagcatgctgaccgccggttatggcagtacccagaccgccagagaacacagcgaccttgtcacaggctatggcagcacttcaacggcagggtcaaacagttcgctgatcgccggctatggaagcactcagacggcgggcttcaaaagcatactgaccgccggttacggcagtacccagacggcacaggagcgcagcgacctggtcgcaggctacggaagcacgtcgactgcgggctattccagttccttgatcgccggctatggcagcacgcagacggcaggctacgaaagcacgttgaccgccggttacggcagtacgcaaaccgctcaggaaaacagctcgctcaccacaggttacggaagtacttctactgcgggctattccagctcgctcatcgcgggttacggcagtacgcaaacggcaggctacgagagcacgttgaccgccggttacggtagtacgcaaaccgcgaaggagcgcagtgatctggtgacaggttatggaagtacctccaccgccggctatgcgagctcgctgattgcgggttatggcagcacgcagactgcgggttatgagagcacgttgaccgccggttacggcagcacgcaaaccgcacaggaaaacagctcgctcaccaccgggtacggaagtacctccacagccggctttgccagctcgctgatcgccggttatggcagtacgcagacagccggctataaaagtaccctcacggccggttacggcagtactcagaccgcagagtatggaagctcactcactgcgggctacggcagcactgcaacggccgggcaggacagttcattgatagccggctatggcagctccctgaccagcggaatcagaagttttctgacggcaggctatggcagtacgctgatcgccggacttcgcagcgttttgatcgccggttatggcagtagtcttacatcgggcgttcgcagcacgttgactgcgggttatggcagtaaccagattgcaagttacggcagctcgttgattgcaggccatgaaagcattcaggtcgccggaaataaaagcatgctgatcgccggcaagggcagctcgcagacagcaggttttcgcagcacgctgattgccggtgcgggcagtgtacaactggcgggtgatcgcagccggttgattgccggtgcagacagtaatcagaccgcgggtgaccgcagcaaactgctggccggtaataacagttatctgactgccggcgatagaagcaaactgaccggcgggcatgactgcaccctgatggcgggagaccaaagcagattgaccgctggtaagaacagtgtcttgacggcaggcgctcgtagcaaactgattggcagtgaaggctcgacgctctcggctggagaagactccatacttattttcaggctctgggacgggaagaggtacaggcaactggtcgccagaacgggtgagaacggtgttgaggccgacataccgtattacgtgaacgaagatgacgatattgtcgataaacccgacgaggacgatgactggatagaggtaaagtag

SEQ ID NO: 3 - protein, 8 aa, Artificial Sequence
  Consensus sequence
AGYGSTLT

SEQ ID NO: 4 - DNA, 30 bp, Artificial Sequence
  Primer P1
gtacgctctagaagtaaacaccctgccggt

SEQ ID NO: 5 - DNA, 69 bp, Artificial Sequence
  Primer P2
aaaaaactgcagttattaatggtgatggtgatggtgagagccggatccctttacctctatccagtcatc

SEQ ID NO: 6 - DNA, 30 bp, Artificial Sequence
  Primer P3
gtaccggaattctttatggtacgctggact

SEQ ID NO: 7 - DNA, 31 bp, Artificial Sequence
  Primer P4
gacccaagcttgcagttattaatggtgatgg

SEQ ID NO: 8 - DNA, 69 bp, Artificial Sequence
  Primer P5
gtaccggaattcactactcatgcaccatcaccatcaccatggatccggctctgtaaacaccctgccggt

SEQ ID NO: 9 - DNA, 34 bp, Artificial Sequence
  Primer P6
aaaaaactgcagactttacctctatccagtcatc

SEQ ID NO: 10 - DNA, 29 bp, Artificial Sequence
  Primer P7
gtaccggaattccatgcaccatcaccatc

SEQ ID NO: 11 - DNA, 30 bp, Artificial Sequence
  Primer P8
gtacgctctagactttgtgagcaattcgtc

SEQ ID NO: 12 - DNA, 64 bp, Artificial Sequence
  Primer P9
aaaaaactgcagaatggtgatggtgatggtgagagccggatccctttacctctatccagtcatc

SEQ ID NO: 13 - DNA, 30 bp, Artificial Sequence
  Primer P10
aacatgccatggctttgtgagcaattcgtc

SEQ ID NO: 14 - protein, 1200 aa, Pseudomonas syringae
MNLDKALVLRTCANNMADHCGLIWPASGTVESRYWQSTRRHENGLVGLLWGAGTSAFLSVHADARWIVCEVAVADIISLEEPGMVKFPRAEVVHVGDRISASHFISARQADPASTSTSTLTPMPTAIPTPMPAVASVTLPVAEQARHEVFDVASVSAAAAPVNTLPVTTPQNVQTATYGSTLSGDNHSRLIAGYGSNETAGNHSDLIAGYGSTGTAGSDSWLVAGYGSTQTAGGDSALTAGYGSTQTAREGSNLTAGYGSTGTAGSDSSLIAGYGSTQTSGGDSSLTAGYGSTQTAQEGSNLTAGYGSTGTAGSDSSLIAGYGSTQTSGGDSSLTAGYGSTQTAQEGSNLTAGYGSTGTAGVDSSLIAGYGSTQTSGSDSALTAGYGSTQTAQEGSNLTAGYGSTGTAGSDSSLIAGYGSTQTSGSDSSLTAGYGSTQTAQEGSILTAGYGSTGTAGVDSSLIAGYGSTQTSGSDSALTAGYGSTQTAQEGSNLTAGYGSTGTAGADSSLIAGYGSTQTSGSESSLTAGYGSTQTAREGSTLTAGYGSTGTAGADSSLIAGYGSTQTSGSESSLTAGYGSTQTAQQGSVLTSGYGSTQTAGAASNLTTGYGSTGTAGHESFIIAGYGSTQTAGHKSILTAGYGSTQTARDGSDLIAGYGSTGTAGSGSSLIAGYGSTQTASYRSMLTAGYGSTQTAREHSDLVTGYGSTSTAGSNSSLIAGYGSTQTAGFKSILTAGYGSTQTAQERTSLVAGYGSTSTAGYSSSLIAGYGSTQTAGYESTLTAGYGSTQTAQENSSLTTGYGSTSTAGYSSSLIAGYGSTQTAGYESTLTAGYGSTQTAQERSDLVTGYGSTSTAGYASSLIAGYGSTQTAGYESTLTAGYGSTQTAQENSSLTTGYGSTSTAGFASSLISGYGSTQTAGYKSTLTAGYGSTQTAEYGSSLTAGYGSTATAGQDSSLIAGYGSSLTSGIRSFLTAGYGSTLIAGLRSVLIAGYGSSLTSGVRSTLTAGYGSNQIASYGSSLIAGHESIQVAGNKSMLIAGKGSSQTAGFRSTLIAGAGSVQLAGDRSRLIAGADSNQTAGDRSKLLAGNNSYLTAGDRSKLTGGHDCTLMAGDQSRLTAGKNSVLTAGARSKLIGSEGSTLSAGEDSILIFRLWDGKRYRQLVARTGENGVEADIPYYVNEDDDIVDKPDEDDDWIEVK

SEQ ID NO: 15 - protein, 1200 aa, Artificial Sequence
  InaZ protein - Clone C4
MNLDKALVLRTCANNMADHCGLIWPASGTVESRYWQSTRRHENGLVGLLWGAGTSAFLSVHADARWIVCEVAVADIISLEEPGMVKFPRAEVVHVGDRISASHFISARQADPASTSTSTLTPMPTAIPTPMPAVASVTLPVAEQARHEVFDVASVSAAAAPVNTLPVTTPQNVQTATYGSTLSGDNHSRLIAGYGSNETAGNHSDLIAGYGSTGTAGSDSWLVAGYGSTQTAGGDSALTAGYGSTQTAREGSNLTAGYGSTGTAGSDSSLIAGYGSTQTSGGDSSLTAGYGSTQTAQEGSNLTAGYGSTGTAGSDSSLIAGYGSTQTSGGDSSLTAGYGSTQTAQEGSNLTAGYGSTGTAGVDSSLIAGYGSTQTSGSDSALTAGYGSTQTAQEGSNLTAGYGSTGTAGSDSSLIAGYGSTQTSGSDSSLTAGYGSTQTAQEGSNLTAGYGSTGTAGVDSSLIAGYGSTQTSGSDSALTAGYGSTQTAQEGSNLTAGYGSTGTAGADSSLIAGYGSTQTSGSESSLTAGYGSTQTAREGSTLTAGYGSTGTAGADSSLIAGYGSTQTSGSESSLTAGYGSTQTAQQGSVLTSGYGSTQTAGAASNLTTGYGSTGTAGHESFIIAGYGSTQTAGHKSILTAGYGSTQTARDGSDLIAGYGSTGTAGSGSSLIAGYGSTQTASYRSMLTAGYGSTQTAREHSDLVTGYGSTSTAGSNSSLIAGYGSTQTAGFKSILTAGYGSTQTAQERSDLVAGYGSTSTAGYSSSLIAGYGSTQTAGYESTLTAGYGSTQTAQENSSLTTGYGSTSTAGYSSSLIAGYGSTQTAGYESTLTAGYGSTQTAKERSDLVTGYGSTSTAGYASSLIAGYGSTQTAGYESTLTAGYGSTQTAQENSSLTTGYGSTSTAGFASSLIAGYGSTQTAGYKSTLTAGYGSTQTAEYGSSLTAGYGSTATAGQDSSLIAGYGSSLTSGIRSFLTAGYGSTLIAGLRSVLIAGYGSSLTSGVRSTLTAGYGSNQIASYGSSLIAGHESIQVAGNKSMLIAGKGSSQTAGFRSTLIAGAGSVQLAGDRSRLIAGADSNQTAGDRSKLLAGNNSYLTAGDRSKLTGGHDCTLMAGDQSRLTAGKNSVLTAGARSKLIGSEGSTLSAGEDSILIFRLWDGKRYRQLVARTGENGVEADIPYYVNEDDDIVDKPDEDDDWIEVK